European Patent Application EP 4 151 655 A1, published March 22, 2023. Title: ANTI-CD25 ANTIBODIES, ANTIGEN-BINDING FRAGMENTS THEREOF, AND MEDICAL USES THEREOF. Applicant: Jiangsu Hengrui Medicine Co., Ltd. Shanghai Shengdi Pharmaceutical Co., Ltd. The sequence listing filed with the application follows.

SEQUENCE LISTING (62 sequences)

SEQ ID NO: 1 - protein, 120 aa, Artificial sequence
  CAB001-VH
QVTLKESGPGILQPSQTLSLTCSFSGFSLNTFGMGVGWIRQPSGKGLEWLAHIWWDDDKYYNPALKSRLTISKDTSKNQVFLKIANVDTADTVTYYCARITTEVGNYDVWGMGTTVTVSS

SEQ ID NO: 2 - protein, 108 aa, Artificial sequence
  CAB001-VL
EIVLTQSPALMAASPGEKVTITCSVSSGITSNNLHWYQQKSETSPKPWIYGTSNLASGVPIRFSGSGSGTSYSLTISSMEAEDAATYYCQQWSSYPFTFGSGTKLEIK

SEQ ID NO: 3 - protein, 120 aa, Artificial sequence
  CAB002-VH
QVTLKESGPGILQPSQTLSLTCSFSGFSLSTFGLGVGWIRQPSGKGLEWLAQIWWDDDEYYNPALKSRLTISKDTSRNQVFLKIANVDTGDTATYFCARMGDTYWYFDVWGTGTTVAVSS

SEQ ID NO: 4 - protein, 108 aa, Artificial sequence
  CAB002-VL
EIVVTQSPALMAVSPGEKVTITCSLSSGITSSNLHWYQQKSETSPKPWIYGTSNLASGVPVRFSGSGSKTSYSLTISSMEAEDAATYYCQQWSSYPFTFGSGTKLEIK

SEQ ID NO: 5 - protein, 121 aa, Artificial sequence
  CAB004-VH
EVQLQQSGAELVRPGASVKLSCTASGFNIKDDYIQWVKQRPEQGLEWIGWIDPENGDTEYASKFQDKATITSDTSSNTAYLQLSSLTSEDTAVYYCAATTFYASNYGFAYWGQGTLVTVSA

SEQ ID NO: 6 - protein, 112 aa, Artificial sequence
  CAB004-VL
DVVMTQTPLSLPVSLGDQASISCRSSQSLVHSNGNTYLHWYLQKPGQSPQLLIYKVSNRFSGVPDRFSGSGSGTDFTLKISRLEAEDLGVYFCSQSTHVPYTFGGGTKLEIK

SEQ ID NO: 7 - protein, 119 aa, Artificial sequence
  CAB006-VH
QIQLQQSGAELMKPGASVKLSCKATGYTFTGHWIEWVKQRPGHGLEWVGEILPGSNKINYNEKFKGKATFTAETSSNTVYMQLSSLTTEDSAIYYCAGGGGPHWPFAFWGQGSLVTVSA

SEQ ID NO: 8 - protein, 111 aa, Artificial sequence
  CAB006-VL
DIVLTQSPASLTVSLGQRATISCRASESVNVHGAHLMHWYQQKPGQPPKLLIYAASILESGVPARFSGSGSETDFTLNIHPVEEEDAATYFCQQTIEDPRTFGGGTKLEIK

SEQ ID NO: 9 - protein, 119 aa, Artificial sequence
  CAB028-VH
EVQLQQSGAELVRPGASVKLSCTASGFNIKNDYVHWVKQRPEQGLEWIGYIDPDNGDTEYASKFLGKATITADTSSNTAYLQLSSLTSEGTAVYYCTTDDTSYGMFACWGLGTLVTVSA

SEQ ID NO: 10 - protein, 112 aa, Artificial sequence
  CAB028-VL
DVLMTQTPLSLPVSLGDQASISCRSSQSIVHSNGNTYLEWYLQKPGQSPKLLIYKVSNRFSGVPDRFSGSGSGTDFTLKISRVEAEDLGVYYCFQGSHVPWTFGGGTKLEIK

SEQ ID NO: 11 - protein, 120 aa, Artificial sequence
  CAB029-VH
QVTLKESGPGILQPSQTLSLTCSFSGFSLSTFGMGVGWIRQPSGKGLEWLAHIWWDDDEYYNPALKSRLTISKDTSKNQVFLKIANVDTADTATYYCTRIMLTTGYFDVWGTGTTVTVSS

SEQ ID NO: 12 - protein, 108 aa, Artificial sequence
  CAB029-VL
EIVLTQSPALMAASPGEKVTITCTVSSGITSSNLHWYQQKSETSPKPWIYGTSNLASGVPVRFSGSGSGTSYSLTISSMEAEDAATYYCQQWSSYPFTFGSGTRLEIK

SEQ ID NO: 13 - protein, 122 aa, Artificial sequence
  CAB037-VH
QVRLQQSGPELVKPGASVQMSCKASGYTFTDYYINWVKQRPGQGLEWIAWIFPGNGNTYFNENFKDKATLSVDKFSSTAFMLLSSLTSEDSAVYFCARATYDHGGYWYFDVWGTGTTVTVSS

SEQ ID NO: 14 - protein, 104 aa, Artificial sequence
  CAB037-VL
QIVLSQSPAILSASPGEKVTMTCRASSSVSHIHWYQQKPGSSPKPWIYATSNLASGVPGRFSGSGSGTSYSLTVSRVEAEDAATYYCQHWNSFTFGGGTELELK

SEQ ID NO: 15 - protein, 119 aa, Artificial sequence
  CAB042-VH
QVQLQQSGPELVKSGASVKLSCKASGYTFTTYDINWMKQRPGQGLEWIGWIYPRDGSTKYNAKFKGKATLTEDTSSNTAFMELHSLTSEDSAVYFCARERIYDGSFDYWGQGTTLTVSS

SEQ ID NO: 16 - protein, 113 aa, Artificial sequence
  CAB042-VL
DIVMTQSPSSLSVSAGEKVSMRCKSSQRLFNSRDQKNYLAWYQQKPGQPPKLLIYGASTRESGVPDRFTGSGSGTDFTLTISSVQAEDLAVYYCQNDHIYPLTFGAGTKLELK

SEQ ID NO: 17 - protein, 116 aa, Artificial sequence
  CAB046-VH
EVQLVESGGGLVKPGGSLKLSCAASGFTFSSYAMSWVRQTPEKRLEWVATISEGGSYTYYPDNVKGRFTISRDNARNNLYLQMSHLKSEDTAMYLCVRDNPWFAYWGQGTLVTVST

SEQ ID NO: 18 - protein, 112 aa, Artificial sequence
  CAB046-VL
DVLMTQTPLSLPVSLGDRASISCRSSQNIVHSNGNTYLEWFLQKPGQSPKLLIYKVSKRFSGVPDRFSGSGSGTDFTLKISRVEAEDLGVYYCFQGSHVPYTFGGGTKLEIK

SEQ ID NO: 19 - protein, 119 aa, Artificial sequence
  PR0006-VH
EVQLVQSGAEVKKPGASVKVSCKASGYTFTGHWIEWVRQAPGQGLEWMGEILPGSNKINYNEKFKGRVTFTADTSTSTVYMELSSLRSEDTAVYYCAGGGGPHWPFAFWGQGTLVTVSS

SEQ ID NO: 20 - protein, 111 aa, Artificial sequence
  PR0006-VL
DIVMTQSPDSLAVSLGERATINCRASESVNVHGAHLMHWYQQKPGQPPKLLIYAASILESGVPDRFSGSGSGTDFTLTISSLQAEDVAVYYCQQTIEDPRTFGGGTKVEIK

SEQ ID NO: 21 - protein, 122 aa, Artificial sequence
  PR0071-VH
EVQLVQSGSELKKPGASVKVSCKASGYTFTDYYINWVRQAPGQGLEWMAWIFPGNGNTYFNENFKDRVTLTADKFSSTAYMELSSLRSEDTAVYYCARATYDHGGYWYFDVWGQGTTVTVSS

SEQ ID NO: 22 - protein, 104 aa, Artificial sequence
  PR0071-VL
EIVLSQSPATLSLSPGERATLSCRASSSVSHIHWYQQKPGSSPKPWIYATSNLASGVPGRFSGSGSGTSYSLTVSRVEAEDAATYYCQHWNSFTFGGGTKVEIK

SEQ ID NO: 23 - protein, 119 aa, Artificial sequence
  PR0031-VH
EVQLVQSGAEVKKPGASVKVSCKASGYTFTTYDINWMKQHPGKGLEWIGWIYPRDGSTKYNAKFKGKATLTEDTSANTAYMELSSLRSEDTAVYYCARERIYDGSFDYWGQGTTVTVSS

SEQ ID NO: 24 - protein, 113 aa, Artificial sequence
  PR0031-VL
DIVMTQSPDSLAVSLGERATINCKSSQRLFNSRDQKNYLAWYQQKPGQPPKLLIYGASTRESGVPDRFSGSGSGTDFTLTISSLQAEDVAVYYCQNDHIYPLTFGQGTKLEIK

SEQ ID NO: 25 - protein, 116 aa, Artificial sequence
  PR0058-VH
EVQLVESGGGLVQPGGSLRLSCAASGFTFSSYAMSWVRQAPGKRLEWVATISEGGSYTYYPDNVKGRFTISRDNSKNTLYLQMNSLRAEDTAVYLCVRDNPWFAYWGQGTLVTVSS

SEQ ID NO: 26 - protein, 112 aa, Artificial sequence
  PR0058-VL
DVLMTQSPLSLPVTPGEPASISCRSSQNIVHSNGNTYLEWFLQKPGQSPKLLIYKVSKRFSGVPDRFSGSGSGTDFTLKISRVEAEDVGVYYCFQGSHVPYTFGGGTKVEIK

SEQ ID NO: 27 - protein, 5 aa, Artificial sequence
  PR0006-HCDR1
GHWIE

SEQ ID NO: 28 - protein, 17 aa, Artificial sequence
  PR0006-HCDR2
EILPGSNKINYNEKFKG

SEQ ID NO: 29 - protein, 10 aa, Artificial sequence
  PR0006-HCDR3
GGGPHWPFAF

SEQ ID NO: 30 - protein, 15 aa, Artificial sequence
  PR0006-LCDR1
RASESVNVHGAHLMH

SEQ ID NO: 31 - protein, 7 aa, Artificial sequence
  PR0006-LCDR2
AASILES

SEQ ID NO: 32 - protein, 9 aa, Artificial sequence
  PR0006-LCDR3
QQTIEDPRT

SEQ ID NO: 33 - protein, 5 aa, Artificial sequence
  PR0071-HCDR1
DYYIN

SEQ ID NO: 34 - protein, 17 aa, Artificial sequence
  PR0071-HCDR2
WIFPGNGNTYFNENFKD

SEQ ID NO: 35 - protein, 13 aa, Artificial sequence
  PR0071-HCDR3
ATYDHGGYWYFDV

SEQ ID NO: 36 - protein, 10 aa, Artificial sequence
  PR0071-LCDR1
RASSSVSHIH

SEQ ID NO: 37 - protein, 7 aa, Artificial sequence
  PR0071-LCDR2
ATSNLAS

SEQ ID NO: 38 - protein, 7 aa, Artificial sequence
  PR0071-LCDR3
QHWNSFT

SEQ ID NO: 39 - protein, 5 aa, Artificial sequence
  PR0031-HCDR1
TYDIN

SEQ ID NO: 40 - protein, 17 aa, Artificial sequence
  PR0031-HCDR2
WIYPRDGSTKYNAKFKG

SEQ ID NO: 41 - protein, 10 aa, Artificial sequence
  PR0031-HCDR3
ERIYDGSFDY

SEQ ID NO: 42 - protein, 17 aa, Artificial sequence
  PR0031-LCDR1
KSSQRLFNSRDQKNYLA

SEQ ID NO: 43 - protein, 7 aa, Artificial sequence
  PR0031-HCDR2
GASTRES

SEQ ID NO: 44 - protein, 9 aa, Artificial sequence
  PR0031-LCDR3
QNDHIYPLT

SEQ ID NO: 45 - protein, 5 aa, Artificial sequence
  PR0058-HCDR1
SYAMS

SEQ ID NO: 46 - protein, 17 aa, Artificial sequence
  PR0058-HCDR2
TISEGGSYTYYPDNVKG

SEQ ID NO: 47 - protein, 7 aa, Artificial sequence
  PR0058-HCDR3
DNPWFAY

SEQ ID NO: 48 - protein, 16 aa, Artificial sequence
  PR0058-LCDR1
RSSQNIVHSNGNTYLE

SEQ ID NO: 49 - protein, 7 aa, Artificial sequence
  PR0058-LCDR2
KVSKRFS

SEQ ID NO: 50 - protein, 9 aa, Artificial sequence
  PR0058-LCDR3
FQGSHVPYT

SEQ ID NO: 51 - protein, 449 aa, Artificial sequence
  PR0006-H
EVQLVQSGAEVKKPGASVKVSCKASGYTFTGHWIEWVRQAPGQGLEWMGEILPGSNKINYNEKFKGRVTFTADTSTSTVYMELSSLRSEDTAVYYCAGGGGPHWPFAFWGQGTLVTVSSASTKGPSVFPLAPSSKSTSGGTAALGCLVKDYFPEPVTVSWNSGALTSGVHTFPAVLQSSGLYSLSSVVTVPSSSLGTQTYICNVNHKPSNTKVDKKVEPKSCDKTHTCPPCPAPELLGGPSVFLFPPKPKDTLMISRTPEVTCVVVDVSHEDPEVKFNWYVDGVEVHNAKTKPREEQYNSTYRVVSVLTVLHQDWLNGKEYKCKVSNKALPAPIEKTISKAKGQPREPQVYTLPPSREEMTKNQVSLTCLVKGFYPSDIAVEWESNGQPENNYKTTPPVLDSDGSFFLYSKLTVDKSRWQQGNVFSCSVMHEALHNHYTQKSLSLSPGK

SEQ ID NO: 52 - protein, 218 aa, Artificial sequence
  PR0006-L
DIVMTQSPDSLAVSLGERATINCRASESVNVHGAHLMHWYQQKPGQPPKLLIYAASILESGVPDRFSGSGSGTDFTLTISSLQAEDVAVYYCQQTIEDPRTFGGGTKVEIKRTVAAPSVFIFPPSDEQLKSGTASVVCLLNNFYPREAKVQWKVDNALQSGNSQESVTEQDSKDSTYSLSSTLTLSKADYEKHKVYACEVTHQGLSSPVTKSFNRGEC

SEQ ID NO: 53 - protein, 452 aa, Artificial sequence
  PR0071-H
EVQLVQSGSELKKPGASVKVSCKASGYTFTDYYINWVRQAPGQGLEWMAWIFPGNGNTYFNENFKDRVTLTADKFSSTAYMELSSLRSEDTAVYYCARATYDHGGYWYFDVWGQGTTVTVSSASTKGPSVFPLAPSSKSTSGGTAALGCLVKDYFPEPVTVSWNSGALTSGVHTFPAVLQSSGLYSLSSVVTVPSSSLGTQTYICNVNHKPSNTKVDKKVEPKSCDKTHTCPPCPAPELLGGPSVFLFPPKPKDTLMISRTPEVTCVVVDVSHEDPEVKFNWYVDGVEVHNAKTKPREEQYNSTYRVVSVLTVLHQDWLNGKEYKCKVSNKALPAPIEKTISKAKGQPREPQVYTLPPSREEMTKNQVSLTCLVKGFYPSDIAVEWESNGQPENNYKTTPPVLDSDGSFFLYSKLTVDKSRWQQGNVFSCSVMHEALHNHYTQKSLSLSPGK

SEQ ID NO: 54 - protein, 211 aa, Artificial sequence
  PR0071-L
EIVLSQSPATLSLSPGERATLSCRASSSVSHIHWYQQKPGSSPKPWIYATSNLASGVPGRFSGSGSGTSYSLTVSRVEAEDAATYYCQHWNSFTFGGGTKVEIKRTVAAPSVFIFPPSDEQLKSGTASVVCLLNNFYPREAKVQWKVDNALQSGNSQESVTEQDSKDSTYSLSSTLTLSKADYEKHKVYACEVTHQGLSSPVTKSFNRGEC

SEQ ID NO: 55 - protein, 449 aa, Artificial sequence
  PR0031-H
EVQLVQSGAEVKKPGASVKVSCKASGYTFTTYDINWMKQHPGKGLEWIGWIYPRDGSTKYNAKFKGKATLTEDTSANTAYMELSSLRSEDTAVYYCARERIYDGSFDYWGQGTTVTVSSASTKGPSVFPLAPSSKSTSGGTAALGCLVKDYFPEPVTVSWNSGALTSGVHTFPAVLQSSGLYSLSSVVTVPSSSLGTQTYICNVNHKPSNTKVDKKVEPKSCDKTHTCPPCPAPELLGGPSVFLFPPKPKDTLMISRTPEVTCVVVDVSHEDPEVKFNWYVDGVEVHNAKTKPREEQYNSTYRVVSVLTVLHQDWLNGKEYKCKVSNKALPAPIEKTISKAKGQPREPQVYTLPPSREEMTKNQVSLTCLVKGFYPSDIAVEWESNGQPENNYKTTPPVLDSDGSFFLYSKLTVDKSRWQQGNVFSCSVMHEALHNHYTQKSLSLSPGK

SEQ ID NO: 56 - protein, 220 aa, Artificial sequence
  PR0031-L
DIVMTQSPDSLAVSLGERATINCKSSQRLFNSRDQKNYLAWYQQKPGQPPKLLIYGASTRESGVPDRFSGSGSGTDFTLTISSLQAEDVAVYYCQNDHIYPLTFGQGTKLEIKRTVAAPSVFIFPPSDEQLKSGTASVVCLLNNFYPREAKVQWKVDNALQSGNSQESVTEQDSKDSTYSLSSTLTLSKADYEKHKVYACEVTHQGLSSPVTKSFNRGEC

SEQ ID NO: 57 - protein, 446 aa, Artificial sequence
  PR0058-H
EVQLVESGGGLVQPGGSLRLSCAASGFTFSSYAMSWVRQAPGKRLEWVATISEGGSYTYYPDNVKGRFTISRDNSKNTLYLQMNSLRAEDTAVYLCVRDNPWFAYWGQGTLVTVSSASTKGPSVFPLAPSSKSTSGGTAALGCLVKDYFPEPVTVSWNSGALTSGVHTFPAVLQSSGLYSLSSVVTVPSSSLGTQTYICNVNHKPSNTKVDKKVEPKSCDKTHTCPPCPAPELLGGPSVFLFPPKPKDTLMISRTPEVTCVVVDVSHEDPEVKFNWYVDGVEVHNAKTKPREEQYNSTYRVVSVLTVLHQDWLNGKEYKCKVSNKALPAPIEKTISKAKGQPREPQVYTLPPSREEMTKNQVSLTCLVKGFYPSDIAVEWESNGQPENNYKTTPPVLDSDGSFFLYSKLTVDKSRWQQGNVFSCSVMHEALHNHYTQKSLSLSPGK

SEQ ID NO: 58 - protein, 219 aa, Artificial sequence
  PR0058-L
DVLMTQSPLSLPVTPGEPASISCRSSQNIVHSNGNTYLEWFLQKPGQSPKLLIYKVSKRFSGVPDRFSGSGSGTDFTLKISRVEAEDVGVYYCFQGSHVPYTFGGGTKVEIKRTVAAPSVFIFPPSDEQLKSGTASVVCLLNNFYPREAKVQWKVDNALQSGNSQESVTEQDSKDSTYSLSSTLTLSKADYEKHKVYACEVTHQGLSSPVTKSFNRGEC

SEQ ID NO: 59 - protein, 116 aa, Artificial sequence
  PR0157-VH
EVQLVESGGGLVQPGGSLRLSCAASGFTFSSYAMSWVRQAPGQRLEWVATISEGGSYTYYPDNVKGRFTISRDNSKNTLYLQMNSLRAEDTAVYLCVRDNPWFAYWGQGTLVTVSS

SEQ ID NO: 60 - protein, 112 aa, Artificial sequence; identical to SEQ ID NO: 26
  PR0157-VL

SEQ ID NO: 61 - protein, 446 aa, Artificial sequence
  PR0157-H
EVQLVESGGGLVQPGGSLRLSCAASGFTFSSYAMSWVRQAPGQRLEWVATISEGGSYTYYPDNVKGRFTISRDNSKNTLYLQMNSLRAEDTAVYLCVRDNPWFAYWGQGTLVTVSSASTKGPSVFPLAPSSKSTSGGTAALGCLVKDYFPEPVTVSWNSGALTSGVHTFPAVLQSSGLYSLSSVVTVPSSSLGTQTYICNVNHKPSNTKVDKKVEPKSCDKTHTCPPCPAPELLGGPSVFLFPPKPKDTLMISRTPEVTCVVVDVSHEDPEVKFNWYVDGVEVHNAKTKPREEQYNSTYRVVSVLTVLHQDWLNGKEYKCKVSNKALPAPIEKTISKAKGQPREPQVYTLPPSREEMTKNQVSLTCLVKGFYPSDIAVEWESNGQPENNYKTTPPVLDSDGSFFLYSKLTVDKSRWQQGNVFSCSVMHEALHNHYTQKSLSLSPGK

SEQ ID NO: 62 - protein, 219 aa, Artificial sequence; identical to SEQ ID NO: 58
  PR0157-L